European Patent Application EP 4 803 110 A1, published September 9, 2026. Title: RECOMBINANT COLLAGEN FILLER, PREPARATION METHOD THEREFOR AND USE THEREOF. Applicant: WitKang Zhiyuan Medical Devices (Xi'an) Co., Ltd. Application EP. The sequence listing filed with the application follows.

SEQUENCE LISTING (1 sequence)

SEQ ID NO: 1 - protein, 399 aa, synthetic construct
GPPGSPGPKGPQGEKGSPGPAGPKGSPGSQGKPGNDGNPGEKGSQGSPGEKGSPGKPGSPGPKGKDGKPGPAGSPGEKGSQGNDGSPGPKGNPGEPGKPGEKGNPGPPGNDGPAGKPGSQGSQGEPGPNGPQGEKGEQGNPGSPGEQGEPGPQGSPGEPGKPGSQGKPGSPGNPGSPGDKGEKGEPGEKGARGNPGPQGPKGANGQPGNPGEKGSQGEPGNPGSQGNPGNPGEPGEKGEKGARGPKGDKGNPGPKGADGSPGKDGKNGEPGSPGKPGPQGEPGDKGNDGPQGPAGSPGEKGEPGDKGARGQPGSPGNQGSQGNDGQPGPKGEPGNDGEKGSQGPPGSPGPQGNPGPQGNDGARGEKGEKGSPGSPGNDGNPGARGKPGSPGPKGNQGKP